European Patent Specification EP 3 438 260 B1, published June 7, 2023. Title: Biomarker of ocular disease. Applicant: Osaka University. The sequence listing filed with the application follows.

SEQUENCE LISTING (6 sequences)

SEQ ID NO: 1 - DNA, 20 bp, Artificial Sequence
  forward primer for cytochrome b
atgaccccaatacgcaaaat

SEQ ID NO: 2 - DNA, 20 bp, Artificial Sequence
  reverse primer for cytochrome b
cgaagtttcatcatgcggag

SEQ ID NO: 3 - DNA, 20 bp, Artificial Sequence
  forward primer for COXIII
atgacccaccaatcacatgc

SEQ ID NO: 4 - DNA, 20 bp, Artificial Sequence
  reverse primer for COXIII
atcacatggctaggccggag

SEQ ID NO: 5 - DNA, 20 bp, Artificial Sequence
  forward primer for NADH
atacccatggccaacctcct

SEQ ID NO: 6 - DNA, 20 bp, Artificial Sequence
  reverse primer for NADH
gggcctttgcgtagttgtat